European Patent Application EP 4 410 829 A1, published August 7, 2024. Title: Protein design using machine learning. Applicant: RevolKa Ltd. The sequence listing filed with the application follows.

SEQUENCE LISTING (9 sequences)

SEQ ID NO: 1 - protein, 116 aa, Lama glama
ELQLVESGGGLVQAGGSLRLSCAASGGTFWRYAMGWFRQAPGKEREFVAHANWSGGRIYYTDSVKGRFTISRDNAKNTVYLQMNSLKPEDTAVYYCRVLSGGRQYWGQGTQVTVSS

SEQ ID NO: 2 - protein, 117 aa, Homo sapiens
EVQLVESGGGLVQPGGSLRLSCAASGFTFSSYAMSWVRQAPGKEREIVSAVSGSGGSTYYADSVKGRFTISRDNSKNTLYLQMNSLRAEDTAVYYCARLKKYAFDYWGQGTLVTVSS

SEQ ID NO: 3 - protein, 116 aa, synthetic construct
EVQLVESGGGLVQPGGSLRLSCAASGGTFWRYAMSWVRQAPGKEREIVSAVNWSGGRTYYADSVKGRFTISRDNSKNTLYLQMNSLRAEDTAVYYCARLSGGRQYWGQGTLVTVSS

SEQ ID NO: 4 - protein, 219 aa, Trichoderma reesei
MQTSCDQWATFTGNGYTVSNNLWGASAGSGFGCVTAVSLSGGASWHADWQWSGGQNNVKSYQNSQIAIPQKRTVNSISSMPTTASWSYSGSNIRANVAYDLFTAANPNHVTYSGDYELMIWLGKYGDIGPIGSSQGTVNVGGQSWTLYYGYNGAMQVYSFVAQTNTTNYSGDVKNFFNYLRDNKGYNAAGQYVLSYQFGTEPFTGSGTLNVASWTASIN

SEQ ID NO: 5 - protein, 116 aa, synthetic construct
EVQLVESGGGLVQPGGSLRLSCAASGGTFWRYAMSWVRQAPGKERELVGASNWSGGRTYYADSVKGRFTISRDNSKNTLYLQMNSLRAEDTAVYYCARLSGGRQYWGQGTLVTVSS

SEQ ID NO: 6 - protein, 116 aa, synthetic construct
EVQLVESGGGLVQPGGSLRLSCAASGGTFWRYAMSWVRQAPGKEREIVGATNWSGGRTYYADSVKGRFTISRDNSKNTLYLQMNSLRAEDTAVYYCARLSGGRQYWGQGTLVTVSS

SEQ ID NO: 7 - protein, 116 aa, synthetic construct
EVQLVESGGGLVQPGGSLRLSCAASGGTFWRYAMSWVRQAPGKERELVGATNWSGGRTYYADSVKGRFTISRDNSKNTLYLQMNSLRAEDTAVYYCARLSGGRQYWGQGTLVTVSS

SEQ ID NO: 8 - protein, 116 aa, synthetic construct
EVQLVESGGGLVQPGGSLRLSCAASGGTFWRYAMSWVRQAPGKEREVVGASNWSGGRTYYADSVKGRFTISRDNSKNTLYLQMNSLRAEDTAVYYCARLSGGRQYWGQGTLVTVSS

SEQ ID NO: 9 - protein, 116 aa
EVQLVESGGGLVQPGGSLRLSCAASGGTFWRYAMSWVRQAPGKEREIVGVSNWSGGRTYYADSVKGRFTISRDNSKNTLYLQMNSLRAEDTAVYYCARLSGGRQYWGQGTLVTVSS